European Patent Application EP 4 177 274 A1, published May 10, 2023. Title: ANTI-FXI/FXIA ANTIBODY, ANTIGEN-BINDING FRAGMENT THEREOF, AND PHARMACEUTICAL USE THEREOF. Applicant: BEIJING TUO JIE BIOPHARMACEUTICAL CO. LTD. Application EP 21832002.6. The sequence listing filed with the application follows.

SEQUENCE LISTING (69 sequences)

SEQ ID NO: 1 - protein, 607 aa, Human (Homo sapiens)
ECVTQLLKDTCFEGGDITTVFTPSAKYCQVVCTYHPRCLLFTFTAESPSEDPTRWFTCVLKDSVTETLPRVNRTAAISGYSFKQCSHQISACNKDIYVDLDMKGINYNSSVAKSAQECQERCTDDVHCHFFTYATRQFPSLEHRNICLLKHTQTGTPTRITKLDKVVSGFSLKSCALSNLACIRDIFPNTVFADSNIDSVMAPDAFVCGRICTHHPGCLFFTFFSQEWPKESQRNLCLLKTSESGLPSTRIKKSKALSGFSLQSCRHSIPVFCHSSFYHDTDFLGEELDIVAAKSHEACQKLCTNAVRCQFFTYTPAQASCNEGKGKCYLKLSSNGSPTKILHGRGGISGYTLRLCKMDNECTTKIKPRIVGGTASVRGEWPWQVTLHTTSPTQRHLCGGSIIGNQWILTAAHCFYGVESPKILRVYSGILNQSEIKEDTSFFGVQEIIIHDQYKMAESGYDIALLKLETTVNYTDSQRPICLPSKGDRNVIYTDCWVTGWGYRKLRDKIQNTLQKAKIPLVTNEECQKRYRGHKITHKMICAGYREGGKDACKGDSGGPLSCKHNEVWHLVGITSWGEGCAQRERPGVYTNVVEYVDWILEKTQAV

SEQ ID NO: 2 - protein, 21 aa, Artificial sequence
  KLH-conjugated FXIa-specific polypeptide
KLHCFYGVESPKILRVYSGIL

SEQ ID NO: 3 - protein, 24 aa, Artificial sequence
  KLH-conjugated FXIa-specific polypeptide
KLHCGYRKLRDKIQNTLQKAKIPL

SEQ ID NO: 4 - protein, 24 aa, Artificial sequence
  KLH-conjugated FXIa-specific polypeptide
KLHCGVQEIIIHDQYKMAESGYDI

SEQ ID NO: 5 - protein, 129 aa, Artificial sequence
  0012-VH
QVQLQQSGAEVKKPGASVKVSCKVSGYTLTELSMHWVRQAPGKGLEWMGGFDPEDGETIYAQKFQGRVTMTEDTSTDTAYMELSSLRSEDTAVYYCATDPHRTWWRYFDWLYPRGMDVWGQGTTVTVSS

SEQ ID NO: 6 - protein, 108 aa, Artificial sequence
  0012-VL
EIVMTQSPGTLSLSPGERATLSCRASQTVGKNYLAWYQQKPGQAPRLLIYGASNRATGIPDRFSGSGSGTDFTLTISRLEPEDFGTYYCQQFRSYPYTFGQGTKVEIK

SEQ ID NO: 7 - protein, 5 aa, Artificial sequence
  0012-HCDR1
ELSMH

SEQ ID NO: 8 - protein, 17 aa, Artificial sequence
  0012-HCDR2
GFDPEDGETIYAQKFQG

SEQ ID NO: 9 - protein, 20 aa, Artificial sequence
  0012-HCDR3
DPHRTWWRYFDWLYPRGMDV

SEQ ID NO: 10 - protein, 12 aa, Artificial sequence
  0012-LCDR1
RASQTVGKNYLA

SEQ ID NO: 11 - protein, 7 aa, Artificial sequence
  0012-LCDR2
GASNRAT

SEQ ID NO: 12 - protein, 9 aa, Artificial sequence
  0012-LCDR3
QQFRSYPYT

SEQ ID NO: 13 - protein, 98 aa, Human (Homo sapiens)
ASTKGPSVFPLAPSSKSTSGGTAALGCLVKDYFPEPVTVSWNSGALTSGVHTFPAVLQSSGLYSLSSVVTVPSSSLGTQTYICNVNHKPSNTKVDKRV

SEQ ID NO: 14 - protein, 107 aa, Human (Homo sapiens) [sequence omitted]

SEQ ID NO: 15 - protein, 459 aa, Artificial sequence
  1209-HC
QVQLQQSGAEVKKPGASVKVSCKVSGYTLTSILMHWVRQAPGKGLEWMGGFDPQDGETVYAQKFQGRVTMTEDTSTDTAYMELSSLRSEDTAVYYCATDPHRTWWRYFDWLYPRGMDVWGQGTTVTVSSASTKGPSVFPLAPSSKSTSGGTAALGCLVKDYFPEPVTVSWNSGALTSGVHTFPAVLQSSGLYSLSSVVTVPSSSLGTQTYICNVNHKPSNTKVDKRVEPKSCDKTHTCPPCPAPELLGGPSVFLFPPKPKDTLMISRTPEVTCVVVDVSHEDPEVKFNWYVDGVEVHNAKTKPREEQYNSTYRVVSVLTVLHQDWLNGKEYKCKVSNKALPAPIEKTISKAKGQPREPQVYTLPPSREEMTKNQVSLTCLVKGFYPSDIAVEWESNGQPENNYKTTPPVLDSDGSFFLYSKLTVDKSRWQQGNVFSCSVMHEALHNHYTQKSLSLSPGK

SEQ ID NO: 16 - protein, 215 aa, Artificial sequence
  1209-LC
EIVMTQSPGTLSLSPGERATLSCRASQTVGKNYLAWYQQKPGQAPRLLIYEASVRALGIPDRFSGSGSGTDFTLTISRLEPEDFGTYYCQQFRSYPYTFGQGTKVEIKRTVAAPSVFIFPPSDEQLKSGTASVVCLLNNFYPREAKVQWKVDNALQSGNSQESVTEQDSKDSTYSLSSTLTLSKADYEKHKVYACEVTHQGLSSPVTKSFNRGEC

SEQ ID NO: 17 - protein, 129 aa, Artificial sequence
  F-VH
QVQLQQSGAEVKKPGASVKVSCKVSGYTLTSIFMHWVRQAPGKGLEWMGGFDPEDGETRYAQKFQGRVTMTEDTSTDTAYMELSSLRSEDTAVYYCATDPHRTWWRYFDWLYPRGMDVWGQGTTVTVSS

SEQ ID NO: 18 - protein, 129 aa, Artificial sequence
  H-VH
QVQLQQSGAEVKKPGASVKVSCKVSGYTLTGLLMHWVRQAPGKGLEWMGGFDPQDGETVYAQKFQGRVTMTEDTSTDTAYMELSSLRSEDTAVYYCATDPHRTWWRYFDWLYPRGMDVWGQGTTVTVSS

SEQ ID NO: 19 - protein, 129 aa, Artificial sequence
  J-VH
QVQLQQSGAEVKKPGASVKVSCKVSGYTLTGVLMHWVRQAPGKGLEWMGGFDPEDGETVYAQKFQGRVTMTEDTSTDTAYMELSSLRSEDTAVYYCATDPHRTWWRYFDWLYPRGMDVWGQGTTVTVSS

SEQ ID NO: 20 - protein, 129 aa, Artificial sequence
  K-VH
QVQLQQSGAEVKKPGASVKVSCKVSGYTLTSILMHWVRQAPGKGLEWMGGFDPQDGETVYAQKFQGRVTMTEDTSTDTAYMELSSLRSEDTAVYYCATDPHRTWWRYFDWLYPRGMDVWGQGTTVTVSS

SEQ ID NO: 21 - protein, 108 aa, Artificial sequence
  3-VL
EIVMTQSPGTLSLSPGERATLSCRASQTVGKNYLAWYQQKPGQAPRLLIYEASVRALGIPDRFSGSGSGTDFTLTISRLEPEDFGTYYCQQFRSYPYTFGQGTKVEIK

SEQ ID NO: 22 - protein, 5 aa, Artificial sequence
  F-VH HCDR1
SIFMH

SEQ ID NO: 23 - protein, 17 aa, Artificial sequence
  F-VH HCDR2
GFDPEDGETRYAQKFQG

SEQ ID NO: 24 - protein, 5 aa, Artificial sequence
  H-VH HCDR1
GLLMH

SEQ ID NO: 25 - protein, 17 aa, Artificial sequence
  H-VH HCDR2
GFDPQDGETVYAQKFQG

SEQ ID NO: 26 - protein, 5 aa, Artificial sequence
  J-VH HCDR1
GVLMH

SEQ ID NO: 27 - protein, 17 aa, Artificial sequence
  J-VH HCDR2
GFDPEDGETVYAQKFQG

SEQ ID NO: 28 - protein, 5 aa, Artificial sequence
  K-VH HCDR1
SILMH

SEQ ID NO: 29 - protein, 7 aa, Artificial sequence
  3-VH LCDR2
EASVRAL

SEQ ID NO: 30 - protein, 129 aa, Artificial sequence
  VH of Fg3g
QVQLVQSGAEVKKPGASVKVSCKVSGYTLTSIFMHWVRQAPGKGLEWMGGFDPEDGETRYAQKFQGRVTMTEDTSTDTAYMELSSLRSEDTAVYYCATDPHRTWWRYFDWLYPRGMDVWGQGTTVTVSS

SEQ ID NO: 31 - protein, 129 aa, Artificial sequence
  VH of Hg3g
QVQLVQSGAEVKKPGASVKVSCKVSGYTLTGLLMHWVRQAPGKGLEWMGGFDPQDGETVYAQKFQGRVTMTEDTSTDTAYMELSSLRSEDTAVYYCATDPHRTWWRYFDWLYPRGMDVWGQGTTVTVSS

SEQ ID NO: 32 - protein, 129 aa, Artificial sequence
  VH of Jg3g
QVQLVQSGAEVKKPGASVKVSCKVSGYTLTGVLMHWVRQAPGKGLEWMGGFDPEDGETVYAQKFQGRVTMTEDTSTDTAYMELSSLRSEDTAVYYCATDPHRTWWRYFDWLYPRGMDVWGQGTTVTVSS

SEQ ID NO: 33 - protein, 129 aa, Artificial sequence
  VH of Kg3g
QVQLVQSGAEVKKPGASVKVSCKVSGYTLTSILMHWVRQAPGKGLEWMGGFDPQDGETVYAQKFQGRVTMTEDTSTDTAYMELSSLRSEDTAVYYCATDPHRTWWRYFDWLYPRGMDVWGQGTTVTVSS

SEQ ID NO: 34 - protein, 108 aa, Artificial sequence
  VL of Fg3g or Hg3g or Jg3g or Kg3g
EIVLTQSPGTLSLSPGERATLSCRASQTVGKNYLAWYQQKPGQAPRLLIYEASVRALGIPDRFSGSGSGTDFTLTISRLEPEDFAVYYCQQFRSYPYTFGQGTKVEIK

SEQ ID NO: 35 - protein, 117 aa, Artificial sequence
  3807-VH
EVQLQQSGAELVRPGTSVKLSCIASGFNIKDDYMHWVKQRPEQGLEWIGWIDPENGDTEYASKFQGKATITADTSANTAYLQFSSLTSEDTAVYYCLYGNFYYFDYWGQGTTLTVSS

SEQ ID NO: 36 - protein, 106 aa, Artificial sequence
  3807-VL
QIVLTQSPAIMSASPGEKVTMTCSASSSINYMHWYQQKPGTSPKRWIYDTSKLASGVPARFSGSGSGTSYSLTISSMEAEDAATYYCHQRSFSPLTFGAGTKLELK

SEQ ID NO: 37 - protein, 5 aa, Artificial sequence
  3807-HCDR1
DDYMH

SEQ ID NO: 38 - protein, 17 aa, Artificial sequence
  3807-HCDR2
WIDPENGDTEYASKFQG

SEQ ID NO: 39 - protein, 8 aa, Artificial sequence
  3807-HCDR3
GNFYYFDY

SEQ ID NO: 40 - protein, 10 aa, Artificial sequence
  3807-LCDR1
SASSSINYMH

SEQ ID NO: 41 - protein, 7 aa, Artificial sequence
  3807-LCDR2
DTSKLAS

SEQ ID NO: 42 - protein, 9 aa, Artificial sequence
  3807-LCDR3
HQRSFSPLT

SEQ ID NO: 43 - protein, 117 aa, Artificial sequence
  3807 VH-CDR grafting
QVQLVQSGAEVKKPGSSVKVSCKASGYTFTDDYMHWVRQAPGQGLEWMGWIDPENGDTEYASKFQGRVTITADESTSTAYMELSSLRSEDTAVYYCARGNFYYFDYWGQGTTVTVSS

SEQ ID NO: 44 - protein, 106 aa, Artificial sequence
  3807 VL-CDR grafting
EIVLTQSPATLSLSPGERATLSCSASSSINYMHWYQQKPGQAPRLLIYDTSKLASGIPARFSGSGSGTDFTLTISSLEPEDFAVYYCHQRSFSPLTFGQGTKLEIK

SEQ ID NO: 45 - protein, 117 aa, Artificial sequence
  3807-VH1
QVQLVQSGAEVKKPGSSVKVSCKASGFNIKDDYMHWVRQAPGQGLEWMGWIDPENGDTEYASKFQGRVTITADESTSTAYMELSSLRSEDTAVYYCLYGNFYYFDYWGQGTTVTVSS

SEQ ID NO: 46 - protein, 117 aa, Artificial sequence
  3807-VH2
QVQLVQSGAEVKKPGSSVKVSCKASGFNIKDDYMHWVRQAPGQGLEWMGWIDPENGDTEYASKFQGRVTITADTSTSTAYMELSSLRSEDTAVYYCLYGNFYYFDYWGQGTTVTVSS

SEQ ID NO: 47 - protein, 117 aa, Artificial sequence
  3807-VH3
QVQLVQSGAEVKKPGSSVKVSCKASGFNIKDDYMHWVRQAPGQGLEWIGWIDPENGDTEYASKFQGRATITADTSTSTAYMELSSLRSEDTAVYYCLYGNFYYFDYWGQGTTVTVSS

SEQ ID NO: 48 - protein, 117 aa, Artificial sequence
  3807-VH4
QVQLVQSGAEVKKPGSSVKVSCKASGFNIKDDYMHWVRQAPGQGLEWIGWIDPENGDTEYASKFQGKATITADTSTSTAYMELSSLRSEDTAVYYCLYGNFYYFDYWGQGTTVTVSS

SEQ ID NO: 49 - protein, 117 aa, Artificial sequence
  3807-VH5
QVQLVQSGAEVKKPGSSVKVSCKASGFNIKDDYMHWVRQAPGQGLEWMGWIDPENGDTEYASKFQGRVTITADTSANTAYMELSSLRSEDTAVYYCLYGNFYYFDYWGQGTTVTVSS

SEQ ID NO: 50 - protein, 106 aa, Artificial sequence
  3807-VL2
EIVLTQSPATLSLSPGERATLSCSASSSINYMHWYQQKPGQAPRLWIYDTSKLASGVPARFSGSGSGTDFTLTISSLEPEDFAVYYCHQRSFSPLTFGQGTKLEIK

SEQ ID NO: 51 - protein, 106 aa, Artificial sequence
  3807-VL3
EIVLTQSPATLSLSPGERATLSCSASSSINYMHWYQQKPGQAPKRWIYDTSKLASGVPARFSGSGSGTDFTLTISSLEPEDFAVYYCHQRSFSPLTFGQGTKLEIK

SEQ ID NO: 52 - protein, 106 aa, Artificial sequence
  3807-VL4
EIVLTQSPATLSLSPGERATLSCSASSSINYMHWYQQKPGQAPRLWIYDTSKLASGVPARFSGSGSGTDYTLTISSLEPEDFAVYYCHQRSFSPLTFGQGTKLEIK

SEQ ID NO: 53 - protein, 117 aa, Artificial sequence
  3807-VH5(ESAN)
QVQLVQSGAEVKKPGSSVKVSCKASGFNIKDDYMHWVRQAPGQGLEWMGWIDPENGDTEYASKFQGRVTITADESANTAYMELSSLRSEDTAVYYCLYGNFYYFDYWGQGTTVTVSS

SEQ ID NO: 54 - protein, 117 aa, Artificial sequence
  3807-VH5(TSTN)
QVQLVQSGAEVKKPGSSVKVSCKASGFNIKDDYMHWVRQAPGQGLEWMGWIDPENGDTEYASKFQGRVTITADTSTNTAYMELSSLRSEDTAVYYCLYGNFYYFDYWGQGTTVTVSS

SEQ ID NO: 55 - protein, 117 aa, Artificial sequence
  3807-VH5(ESTN)
QVQLVQSGAEVKKPGSSVKVSCKASGFNIKDDYMHWVRQAPGQGLEWMGWIDPENGDTEYASKFQGRVTITADESTNTAYMELSSLRSEDTAVYYCLYGNFYYFDYWGQGTTVTVSS

SEQ ID NO: 56 - protein, 117 aa, Artificial sequence
  3807-VH1(AR)
QVQLVQSGAEVKKPGSSVKVSCKASGFNIKDDYMHWVRQAPGQGLEWMGWIDPENGDTEYASKFQGRVTITADESTSTAYMELSSLRSEDTAVYYCARGNFYYFDYWGQGTTVTVSS

SEQ ID NO: 57 - protein, 117 aa, Artificial sequence
  3807-VH1(YTFT)
QVQLVQSGAEVKKPGSSVKVSCKASGYTFTDDYMHWVRQAPGQGLEWMGWIDPENGDTEYASKFQGRVTITADESTSTAYMELSSLRSEDTAVYYCLYGNFYYFDYWGQGTTVTVSS

SEQ ID NO: 58 - protein, 117 aa, Artificial sequence
  3807-VH1(GTFS)
QVQLVQSGAEVKKPGSSVKVSCKASGGTFSDDYMHWVRQAPGQGLEWMGWIDPENGDTEYASKFQGRVTITADESTSTAYMELSSLRSEDTAVYYCLYGNFYYFDYWGQGTTVTVSS

SEQ ID NO: 59 - protein, 98 aa, Artificial sequence
  Heavy chain CH1 of human antibody
ASTKGPSVFPLAPCSRSTSESTAALGCLVKDYFPEPVTVSWNSGALTSGVHTFPAVLQSSGLYSLSSVVTVPSSSLGTKTYTCNVDHKPSNTKVDKRV

SEQ ID NO: 60 - protein, 229 aa, Artificial sequence
  IgG4PFc (containing the S241P mutation) of human antibody
ESKYGPPCPPCPAPEFLGGPSVFLFPPKPKDTLMISRTPEVTCVVVDVSQEDPEVQFNWYVDGVEVHNAKTKPREEQFNSTYRVVSVLTVLHQDWLNGKEYKCKVSNKGLPSSIEKTISKAKGQPREPQVYTLPPSQEEMTKNQVSLTCLVKGFYPSDIAVEWESNGQPENNYKTTPPVLDSDGSFFLYSRLTVDKSRWQEGNVFSCSVMHEALHNHYTQKSLSLSLGK

SEQ ID NO: 61 - protein, 444 aa, Artificial sequence
  3882-HC
QVQLVQSGAEVKKPGSSVKVSCKASGGTFSDDYMHWVRQAPGQGLEWMGWIDPENGDTEYASKFQGRVTITADESTSTAYMELSSLRSEDTAVYYCLYGNFYYFDYWGQGTTVTVSSASTKGPSVFPLAPCSRSTSESTAALGCLVKDYFPEPVTVSWNSGALTSGVHTFPAVLQSSGLYSLSSVVTVPSSSLGTKTYTCNVDHKPSNTKVDKRVESKYGPPCPPCPAPEFLGGPSVFLFPPKPKDTLMISRTPEVTCVVVDVSQEDPEVQFNWYVDGVEVHNAKTKPREEQFNSTYRVVSVLTVLHQDWLNGKEYKCKVSNKGLPSSIEKTISKAKGQPREPQVYTLPPSQEEMTKNQVSLTCLVKGFYPSDIAVEWESNGQPENNYKTTPPVLDSDGSFFLYSRLTVDKSRWQEGNVFSCSVMHEALHNHYTQKSLSLSLGK

SEQ ID NO: 62 - protein, 213 aa, Artificial sequence
  3882-LC
EIVLTQSPATLSLSPGERATLSCSASSSINYMHWYQQKPGQAPKRWIYDTSKLASGVPARFSGSGSGTDFTLTISSLEPEDFAVYYCHQRSFSPLTFGQGTKLEIKRTVAAPSVFIFPPSDEQLKSGTASVVCLLNNFYPREAKVQWKVDNALQSGNSQESVTEQDSKDSTYSLSSTLTLSKADYEKHKVYACEVTHQGLSSPVTKSFNRGEC

SEQ ID NO: 63 - protein, 5 aa, Artificial sequence
  General formula of HCDR1
  VARIANT (1)..(1): Xaa is selected from the group consisting of E, S, G and D
  VARIANT (2)..(2): Xaa is selected from the group consisting of L, I, V and D
  VARIANT (3)..(3): Xaa is selected from the group consisting of S, F, L and Y
XXXMH

SEQ ID NO: 64 - protein, 17 aa, Artificial sequence
  General formula of HCDR2
  VARIANT (1)..(1): Xaa is selected from the group consisting of G and W
  VARIANT (2)..(2): Xaa is selected from the group consisting of F and I
  VARIANT (5)..(5): Xaa is selected from the group consisting of E and Q
  VARIANT (6)..(6): Xaa is selected from the group consisting of D and N
  VARIANT (8)..(8): Xaa is selected from the group consisting of E and D
  VARIANT (10)..(10): Xaa is selected from the group consisting of I, R, V and E
  VARIANT (13)..(13): Xaa is selected from the group consisting of Q and S
XXDPXXGXTXYAXKFQG

SEQ ID NO: 65 - protein, 7 aa, Artificial sequence
  General formula of LCDR2
  VARIANT (1)..(1): Xaa is selected from the group consisting of G, E and D
  VARIANT (2)..(2): Xaa is selected from the group consisting of A and T
  VARIANT (4)..(4): Xaa is selected from the group consisting of N, V and K
  VARIANT (5)..(5): Xaa is selected from the group consisting of R and L
  VARIANT (7)..(7): Xaa is selected from the group consisting of T, L and S
XXSXXAX

SEQ ID NO: 66 - protein, 9 aa, Artificial sequence
  General formula of LCDR3
  VARIANT (1)..(1): Xaa is selected from the group consisting of Q and H
  VARIANT (3)..(3): Xaa is selected from the group consisting of F and R
  VARIANT (4)..(4): Xaa is selected from the group consisting of R and S
  VARIANT (5)..(5): Xaa is selected from the group consisting of S and F
  VARIANT (6)..(6): Xaa is selected from the group consisting of Y and S
  VARIANT (8)..(8): Xaa is selected from the group consisting of Y and L
XQXXXXPXT

SEQ ID NO: 67 - protein, 232 aa, Human (homo sapiens)
EPKSCDKTHTCPPCPAPELLGGPSVFLFPPKPKDTLMISRTPEVTCVVVDVSHEDPEVKFNWYVDGVEVHNAKTKPREEQYNSTYRVVSVLTVLHQDWLNGKEYKCKVSNKALPAPIEKTISKAKGQPREPQVYTLPPSREEMTKNQVSLTCLVKGFYPSDIAVEWESNGQPENNYKTTPPVLDSDGSFFLYSKLTVDKSRWQQGNVFSCSVMHEALHNHYTQKSLSLSPGK

SEQ ID NO: 68 - protein, 449 aa, Artificial sequence
  Heavy chain of BAY1213790
EVQLLESGGGLVQPGGSLRLSCAASGFTFSQYGMDWVRQAPGKGLEWVSGIGPSGGSTVYADSVKGRFTISRDNSKNTLYLQMNSLRAEDTAVYYCTRGGPYYYYGMDVWGQGTTVTVSSASTKGPSVFPLAPSSKSTSGGTAALGCLVKDYFPEPVTVSWNSGALTSGVHTFPAVLQSSGLYSLSSVVTVPSSSLGTQTYICNVNHKPSNTKVDKKVEPKSCDKTHTCPPCPAPELLGGPSVFLFPPKPKDTLMISRTPEVTCVVVDVSHEDPEVKFNWYVDGVEVHNAKTKPREEQYNSTYRVVSVLTVLHQDWLNGKEYKCKVSNKALPAPIEKTISKAKGQPREPQVYTLPPSRDELTKNQVSLTCLVKGFYPSDIAVEWESNGQPENNYKTTPPVLDSDGSFFLYSKLTVDKSRWQQGNVFSCSVMHEALHNHYTQKSLSLSPG

SEQ ID NO: 69 - protein, 214 aa, Artificial sequence
  Light chain of BAY1213790
DIQMTQSPSSLSASVGDRVTITCQASQDISNYLNWYQQKPGKAPKLLIYDASNLETGVPSRFSGSGSGTDFTFTISSLQPEDIATYYCQQADSFPVTFGGGTKVEIKRTVAAPSVFIFPPSDEQLKSGTASVVCLLNNFYPREAKVQWKVDNALQSGNSQESVTEQDSKDSTYSLSSTLTLSKADYEKHKVYACEVTHQGLSSPVTKSFNRGEC